European Patent Application EP 4 130 239 A1, published February 8, 2023. Title: Method for inducing differentiation into pancreatic  ¿ cells. Applicant: KANEKA CORPORATION National Center for Global Health and Medicine. The sequence listing filed with the application follows.

SEQUENCE LISTING (12 sequences)

SEQ ID NO: 1 - DNA, 24 bp, Artificial Sequence
  Forward primer
gtcagagggatcacaatctttcag

SEQ ID NO: 2 - DNA, 23 bp, Artificial Sequence
  Riverse primer
gtcttgtcgttggacgttagttc

SEQ ID NO: 3 - DNA, 20 bp, Artificial Sequence
  Forward primer
ttgtgaaccaacacctgtgc

SEQ ID NO: 4 - DNA, 23 bp, Artificial Sequence
  Riverse primer
gtgtgtagaagaagcctcgttcc

SEQ ID NO: 5 - DNA, 24 bp, Artificial Sequence
  Forward primer
acattcaccagtgactacagcaag

SEQ ID NO: 6 - DNA, 22 bp, Artificial Sequence
  Riverse primer
ggcaatgttattcctgttcctc

SEQ ID NO: 7 - DNA, 20 bp, Artificial Sequence
  Forward primer
atcttcgccctggagaagac

SEQ ID NO: 8 - DNA, 20 bp, Artificial Sequence
  Riverse primer
cgtgcttcttcctccacttg

SEQ ID NO: 9 - DNA, 21 bp, Artificial Sequence
  Forward primer
aaggaggtgtgctaaaggctg

SEQ ID NO: 10 - DNA, 22 bp, Artificial Sequence
  Riverse primer
gctggtcctctgtttccatttg

SEQ ID NO: 11 - DNA, 20 bp, Artificial Sequence
  Forward primer
ctgagtgctgcaccaaagag

SEQ ID NO: 12 - DNA, 23 bp, Artificial Sequence
  Riverse primer
atttgtgggttccacgtaggtag